European Patent Application EP 4 729 614 A1, published April 22, 2026. Title: 分离mRNA的系统和方法. Applicant: 苏州艾博生物科技有限公司. Application CN. The sequence listing filed with the application follows.

SEQUENCE LISTING (20 sequences)

SEQ ID NO: 1 - RNA, 1075 nt, synthetic construct
  source 1..1075: mol_type = other RNA
ggggggatccaagcttagcttgcttgttctttttgcagaagctcagaataaacgctcaactttggcgccgccaccatggactggacctggattctcttcttggtggcagcagccacgcgagtccactccagagtgcagcctaccgagagcatcgtgagattccctaatatcaccaatctgtgccctttcggcgaggtgttcaatgccaccagattcgccagcgtgtacgcatggaaccgcaagcggataagcaattgcgtggccgactacagcgtgctgtacaatagcgccagcttcagcaccttcaaatgttatggtgtttcgccaacaaagctgaatgacctgtgcttcaccaatgtgtacgccgacagcttcgtgatcagaggcgacgaggtgagacagatcgcgccagggcagaccggcaagatcgccgactacaattacaagctgcctgacgacttcaccggctgcgtgatcgcgtggaactctaacaatctagattcgaaagttggaggcaattacaattaccggtacagactgttcagaaagagcaatctgaagcctttcgagagagacatcagcaccgagatctaccaggccggcagcaaaccgtgtaatggcgtggagggcttcaattgctacttccctctgcagagctacggcttccagcctaccaatggcgtgggctaccagccttacagagtggtggtgctgagcttcgagctgctgcacgctcccgctaccgtgtgcggccctaagaagagcaccaatctggtgaagaataagtgcgtgaatttctgataagaattctaggctggagcctcggtggccatgcttcttgccccttgggcctccccccagcccctcctccccttcctgcacccgtacccccgtggtctttgaataaagtctgagtgggcggcactagtaaaaaaaaaaaaaaaaaaaaaaaaaaaaaaaaaaaaaaaaaaaaaaaaaaaaaaaaaaaaaaaaaaaaaaaaaaaaaaaaaaaaaaaaaaaaaaaaaaaaaaaaaaaaaaaaaaaaaaaaaaaaaaaaaaaaaaaaaaaaaaaaaa

SEQ ID NO: 2 - RNA, 985 nt, synthetic construct
  source 1..985: mol_type = other RNA
ggggggatccgcaggagccagggctgggcataaaagtcagggcagagccatctattgcttacatttgcttctgacacaactgtgttcactagcaacctcaaacagacaccatgggggtgcacgaatgtcctgcctggctgtggcttctcctgtccctgctgtcgctccctctgggcctcccagtcctgggcgccccaccacgcctcatctgtgacagccgagtcctggagaggtacctcttggaggccaaggaggccgagaatatcacgacgggctgtgctgaacactgcagcttgaatgagaatatcactgtcccagacaccaaagttaatttctatgcctggaagaggatggaggtcgggcagcaggccgtagaagtctggcagggcctggccctgctgtcggaagctgtcctgcggggccaggccctgttggtcaactcttcccagccgtgggagcccctgcagctgcatgtggataaagccgtcagtggccttcgcagcctcaccactctgcttcgggctctgggagcccagaaggaagccatctcccctccagatgcggcctcagctgctccactccgaacaatcactgctgacactttccgcaaactcttccgagtctactccaatttcctccggggaaagctgaagctgtacacaggggaggcctgcaggacaggggacagatgataagaattcgctcgctttcttgctgtccaatttctattaaaggttcctttgttccctaagtccaactactaaactgggggatattatgaagggccttgagcatctggattctgcctaataaaaaacatttattttcattgcactagtaaaaaaaaaaaaaaaaaaaaaaaaaaaaaaaaaaaaaaaaaaaaaaaaaaaaaaaaaaaaaaaaaaaaaaaaaaaaaaaaaaaaaaaaaaaaaaaaaaaaaaaaaaaaaaaaaaaaaaaaaaaaaaaaaaaaaaaaaaaaaaaaaa

SEQ ID NO: 3 - RNA, 1069 nt, synthetic construct
  source 1..1069: mol_type = other RNA
ggggggatccaagcttagcttgcttgttctttttgcagaagctcagaataaacgctcaactttggcgccgccaccatggtgagcaagggcgaggagctgttcaccggggtggtgcccatcctggtcgagctggacggcgacgtaaacggccacaagttcagcgtgtccggcgagggcgagggcgatgccacctacggcaagctgaccctgaagttcatctgcaccaccggcaagctgcccgtgccctggcccaccctcgtgaccaccctgacctacggcgtgcagtgcttcagccgctaccccgaccacatgaagcagcacgacttcttcaagtccgccatgcccgaaggctacgtccaggagcgcaccatcttcttcaaggacgacggcaactacaagacccgcgccgaggtgaagttcgagggcgacaccctggtgaaccgcatcgagctgaagggcatcgacttcaaggaggacggcaacatcctggggcacaagctggagtacaactacaacagccacaacgtctatatcatggccgacaagcagaagaacggcatcaaggtgaacttcaagatccgccacaacatcgaggacggcagcgtgcagctcgccgaccactaccagcagaacacccccatcggcgacggccccgtgctgctgcccgacaaccactacctgagcacccagtccgccctgagcaaagaccccaacgagaagcgcgatcacatggtcctgctggagttcgtgaccgccgccgggatcactctcggcatggacgagctgtacaagtgataagaattctaggctggagcctcggtggccatgcttcttgccccttgggcctccccccagcccctcctccccttcctgcacccgtacccccgtggtctttgaataaagtctgagtgggcggcactagtaaaaaaaaaaaaaaaaaaaaaaaaaaaaaaaaaaaaaaaaaaaaaaaaaaaaaaaaaaaaaaaaaaaaaaaaaaaaaaaaaaaaaaaaaaaaaaaaaaaaaaaaaaaaaaaaaaaaaaaaaaaaaaaaaaaaaaaaaaaaaaaaaa

SEQ ID NO: 4 - RNA, 1996 nt, synthetic construct
  source 1..1996: mol_type = other RNA
ggggggatccaagcttagcttgcttgttctttttgcagaagctcagaataaacgctcaactttggcgccgccaccatggaagatgcgaagaacatcaagaagggacctgccccgttttaccctttggaggacggtacagcaggagaacagctccacaaggcgatgaaacgctacgccctggtccccggaacgattgcgtttaccgatgcacatattgaggtagacatcacatacgcagaatacttcgaaatgtcggtgaggctggcggaagcgatgaagagatatggtcttaacactaatcaccgcatcgtggtgtgttcggagaactcattgcagtttttcatgccggtccttggagcacttttcatcggggtcgcagtcgcgccagcgaacgacatctacaatgagcgggaactcttgaatagcatgggaatctcccagccgacggtcgtgtttgtctccaaaaaggggctgcagaaaatcctcaacgtgcagaagaagctccccattattcaaaagatcatcattatggatagcaagacagattaccaagggttccagtcgatgtatacctttgtgacatcgcatttgccgccagggtttaacgagtatgacttcgtccccgagtcatttgacagagataaaaccatcgcgctgattatgaactcctcgggtagcaccggtttgccaaagggggtggcgttgccccaccgcactgcttgtgtgcggttctcgcacgctagggaccctatctttggtaatcagatcattcccgacacagcaatcctgtccgtggtaccttttcatcacggttttggcatgttcacgactctcggctatttgatttgcggtttcagggtcgtacttatgtatcggttcgaggaagaactgtttttgagatccttgcaagattacaagatccagtcggccctccttgtgccaacgcttttctcattctttgcgaaatcgacacttattgataagtatgacctttccaatctgcatgagattgcctcagggggagcgccgcttagcaaggaagtcggggaggcagtggccaagcgcttccaccttcccggaatccggcagggatacgggctcacggagacaacatccgcgatccttatcacgcccgagggtgacgataagccgggagccgtcggaaaagtggtccccttctttgaagccaaggtcgtagacctcgacacgggaaaaaccctcggagtgaaccagaggggcgagctctgcgtgagagggccgatgatcatgtcaggttacgtgaataaccctgaagcgacgaatgcgctgatcgacaaggatgggtggttgcattcgggagacattgcctattgggatgaggatgagcacttctttatcgtagatcgacttaagagcttgatcaaatacaaaggctatcaggtagcgcctgccgagctcgagtcaatcctgctccagcaccccaacattttcgacgccggagtggccgggttgcccgatgacgacgcgggtgagctgccagcggccgtggtagtcctcgaacatgggaaaacaatgaccgaaaaggagatcgtggactacgtagcatcacaagtgacgactgcgaagaaactgaggggaggggtagtctttgtggacgaggtcccgaaaggcttgactgggaagcttgacgctcgcaaaatccgggaaatcctgattaaggcaaagaaaggcgggaaaatcgctgtctgataataggctggagcctcggtggccatgcttcttgccccttgggcctccccccagcccctcctccccttcctgcacccgtacccccgtggtctttgaataaagtctgagtgggcggcactagtaaaaaaaaaaaaaaaaaaaaaaaaaaaaaaaaaaaaaaaaaaaaaaaaaaaaaaaaaaaaaaaaaaaaaaaaaaaaaaaaaaaaaaaaaaaaaaaaaaaaaaaaaaaaaaaaaaaaaaaaaaaaaaaaaaaaaaaaaaaaaaaaaa

SEQ ID NO: 5 - RNA, 1075 nt, synthetic construct
  source 1..1075: mol_type = other RNA
ggggggatccaagcttagcttgcttgttctttttgcagaagctcagaataaacgctcaactttggcgccgccaccatggactggacctggattctcttcttggtggcagcagccacgcgagtccactccagagtccaaccaacagaatctattgttagatttcctaatattacaaacttgtgcccttttggtgaagtttttaacgccaccagatttgcatctgtttatgcttggaacaggaagagaatcagcaactgtgttgctgattattctgtcctatataattccgcatcattttccacttttaagtgttatggagtgtctcctactaaattaaatgatctctgctttactaatgtctatgcagattcatttgtaattagaggtgatgaagtcagacaaatcgctccagggcaaactggaaagattgctgattataattataaattaccagatgattttacaggctgcgttatagcttggaactctaacaatcttgattctaaggttggtggtaattataattacctgtatagattgtttaggaagtctaatctcaaaccttttgagagagatatttcaactgaaatctatcaggccggtagcacaccttgtaatggtgttgaaggttttaattgttactttcctttacaatcatatggtttccaacccactaatggtgttggttaccaaccatacagagtagtagtactttcttttgaacttctacatgcaccagcaactgtttgtggacctaaaaagtctactaatttggttaaaaacaaatgtgtcaatttctgataagaattctaggctggagcctcggtggccatgcttcttgccccttgggcctccccccagcccctcctccccttcctgcacccgtacccccgtggtctttgaataaagtctgagtgggcggcactagtaaaaaaaaaaaaaaaaaaaaaaaaaaaaaaaaaaaaaaaaaaaaaaaaaaaaaaaaaaaaaaaaaaaaaaaaaaaaaaaaaaaaaaaaaaaaaaaaaaaaaaaaaaaaaaaaaaaaaaaaaaaaaaaaaaaaaaaaaaaaaaaaaa

SEQ ID NO: 6 - RNA, 1973 nt, synthetic construct
  source 1..1973: mol_type = other RNA
ggggggatccaagcttagcttgcttgttctttttgcagaagctcagaataaacgctcaactttggcgccgccaccatgtgtcctcagaagctaaccatctcctggtttgccatcgttttgctggtgtctccactcatggccatgtgggagctggagaaagacgtttatgttgtagaggtggactggactcccgatgcccctggagaaacagtgaacctcacctgtgacacgcctgaagaagatgacatcacctggacctcagaccagagacatggagtcataggctctggaaagaccctgaccatcactgtcaaagagttcctagatgctggccagtacacctgccacaaaggaggcgagactctgagccactcacatctgctgctccacaagaaggaaaatggaatttggtccactgaaattttaaaaaatttcaaaaacaagactttcctgaagtgtgaagcaccaaattactccggacggttcacgtgctcatggctggtgcaaagaaacatggacttgaagttcaacatcaagagcagtagcagttcccctgactctcgggcagtgacatgtggaatggcgtctctgtctgcagagaaggtcacactggaccaaagggactatgagaagtattcagtgtcctgccaggaggatgtcacctgcccaactgccgaggagacactgcccattgaactggcgttggaagcacggcagcagaataaatatgagaactacagcaccagcttcttcatcagggacatcatcaaaccagacccgcccaagaacttgcagatgaagcctttgaagaactcacaggtggaggtcagctgggagtaccctgactcctggagcactccccattcctacttctccctcaagttctttgttcgaatccagcgcaagaaagaaaagatgaggagacagaggaggggtgtaaccagaaaggtgcgttcctcgtagagaagacatctaccgaagtccaatgcaaaggcgggaatgtctgcgtgcaagctcaggatcgctattacaattcctcatgcagcaagtgggcatgtgttccctgcagggtccgatccggaggcgggggagcggaggcggagggagcggaggcggagggagcagggtcattccagtctctggacctgccaggtgtcttagccagtcccgaaacctgctgaagaccacagatgacatggtgaagacggccagagaaaaactgaaacattattcctgcactgctgaagacatcgatcatgaagacatcacacgggaccaaaccagcacattgaagacctgtttaccactggaactacacaagaacgagagttgcctggctactagagagacttcttccacaacaagagggagctgcctgcccccacagaagacgtctttgatgatgaccctgtgccttggtagcatctatgaggacttgaagatgtaccagacagagttccaggccatcaacgcagcacttcagaatcacaaccatcagcagatcattttagacaagggcatgctggtggccatcgatgagctgatgcagtctctgaatcataatggcgagactctgcgccagaaacctcctgtgggagaagcagacccttacagagtgaaaatgaagctctgcatcctgcttcacgccttcagcacccgcgtcgtgaccatcaacagggtgatgggctatctgagctccgcctgataataggctggagcctcggtggccatgcttcttgccccttgggcctccccccagcccctcctccccttcctgcacccgtacccccgtggtctttgaataaagtctgagtgggcggcactagtaaaaaaaaaaaaaaaaaaaaaaaaaaaaaaaaaaaaaaaaaaaaaaaaaaaaaaaaaaaaaaaaaaaaaaaaaaaaaaaaaaaaaaaaaaaaaaaaaaaaaaaaaaaaaaaaaaaaaaaaaaaaaaaaaaaaaaaaaaaaaaaaaa

SEQ ID NO: 7 - RNA, 2050 nt, synthetic construct
  source 1..2050: mol_type = other RNA
ggggggatccaagcttagcttgcttgttctttttgcagaagctcagaataaacgctcaactttggcgccgccaccatgaaagccatcctggtggtaatgctgtacaccttcaccacagccaacgccgacaccctgtgcatcggctaccacgccaacaacagcaccgacaccgtggacaccgtgctagagaaaaacgtgaccgtgacccacagcgtgaacctgctggaggacaaacacaacggcaaactgtgcaaactgagaggcgtggcacccctgcacctgggcaaatgcaacatcgccggctggatactgggaaaccccgagtgcgagagcctgagcaccgccaggagctggagctacatcgtggagacaagcaacagcgacaacggcacctgctacccaggcgacttcatcaactacgaggagctgcgagagcagctcagcagcgtgagcagcttcgagcgcttcgaaatcttccccaaaacaagcagctggccaaaccacgacagcgacaacggcgtgaccgccgcctgcccccacgccggcgccaaaagtttctacaaaaacctgatctggctggtgaaaaaaggcaaaagctaccccaaaatcaaccagacctacatcaacgacaaaggcaaagaggtgctcgtgctgtggggcatccaccacccgcccaccatcgcagaccagcagagcctgtaccagaacgccgacgcctacgtgttcgtgggcaccagccggtacagcaaaaaattcaaacccgagatcgccaccagacccaaagtgagggaccaggagggcagaatgaactactactggaccctggtggagcccggcgacaaaatcaccttcgaggccaccgggaacctggtggcacccagatacgccttcacaatggagagagacgccggcagcggcatcatcatcagcgacacccccgtgcacgactgcaacaccacctgccagacccccgaaggcgccatcaacaccagcctgcccttccagaacgtacacccaatcaccatcggcaaatgccccaaatacgtgaaaagcaccaaactgagactggccaccggcctgaggaacgtgcccagcatccagagcaggggcctgttcggcgccatcgccggcttcatcgagggcggctggaccggcatggtggacggctggtacggctaccaccaccagaacgagcaggggagcggctacgccgccgacctgaaaagcacacagaacgccatcgacaaaatcaccaacaaagtgaacagcgtgatagagaaaatgaacacccagttcaccgccgtgggcaaagagttcaaccacctggagaaaagaatcgagaacctgaacaaaaaagtggacgacggcttcctggacatctggacctacaacgccgagctgctggtgctgctggagaacgagagaaccctggactaccacgacagcaacgtgaaaaacctgtacgagaaagtgcggaaccagctgaaaaacaacgccaaagagatcgggaacgggtgcttcgagttctaccacaaatgcgacaacacctgcatggagagcgtgaaaaacggcacctacgactaccccaaatacagcgaggaggccaaactgaacagagagaaaatcgacggagtcaaactggacagcaccagaatctaccagatcctggcaatctacagcaccgtggccagcagcctggtgctggtggtgagcctgggcgccatcagcttctggatgtgcagcaacggcagcctccagtgcagaatctgcatatgataagaattctaggctggagcctcggtggccatgcttcttgccccttgggcctccccccagcccctcctccccttcctgcacccgtacccccgtggtctttgaataaagtctgagtgggcggcactagtaaaaaaaaaaaaaaaaaaaaaaaaaaaaaaaaaaaaaaaaaaaaaaaaaaaaaaaaaaaaaaaaaaaaaaaaaaaaaaaaaaaaaaaaaaaaaaaaaaaaaaaaaaaaaaaaaaaaaaaaaaaaaaaaaaaaaaaaaaaaaaaaaa

SEQ ID NO: 8 - RNA, 2050 nt, synthetic construct
  source 1..2050: mol_type = other RNA
ggggggatccaagcttagcttgcttgttctttttgcagaagctcagaataaacgctcaactttggcgccgccaccatgaagaccatcatcgctctgagcaacatcctgtgcctggtgttcgcccagaagatccctggcaacgacaactccaccgccaccctgtgcctgggccaccacgccgtgcccaacggcaccatcgtgaagaccatcaccaacgacaggatcgaggtgaccaatgccaccgagctggtgcagaactcctccatcggggagatctgcggcagcccccaccagatcctggatgggggcaattgcaccctgatcgacgccctgctgggcgatcctcagtgtgatggcttccagaataaggagtgggacctgttcgtggagaggagcagagctaacagcaactgctacccctacgacgtgcccgactacgcctccctgaggagcctggtggccagcagcgggaccctggagttcaagaacgagagcttcaattggaccggcgtgaagcagaatggcaccagctctgcctgcatcagagggagcagcagctccttcttcagcaggctgaattggctgaccagcctgaacaatatctaccctgcccagaacgtgaccatgcctaacaaggagcagtttgacaagctgtacatctggggggtgcaccaccccgacaccgacaagaatcagatctctctgttcgcccagagctccggcaggatcaccgtgagcaccaagaggagccagcaggccgtgatccccaacatcggcagccggccccggatcagggacatccctagccggatcagcatctactggaccatcgtgaagcccggcgacatcctgctgatcaattccaccggcaatctgatcgcccccaggggctacttcaagatccggtccggcaagagcagcatcatgaggagcgacgcccccatcgggaagtgcaagtctgagtgcatcacccccaacgggagcatccccaatgataagcccttccagaacgtgaaccggatcacttacggggcctgcccacggtacgtgaagcagagcaccctgaagctggccaccgggatgaggaatgtgcccgagaagcagaccagaggcatcttcggcgccatcgccggcttcatcgagaacggctgggagggcatggtggacggctggtacggcttccggcaccagaactctgagggccggggccaggccgccgacctgaagagcacccaggccgccattgatcagatcaatggcaagctgaaccggctgatcgggaagaccaacgagaagttccaccagatcgagaaggagttcagcgaggtggagggcagggtgcaggacctggagaagtacgtggaggacaccaagatcgacctgtggagctacaacgccgagctgctggtggccctggagaaccagcacaccatcgacctgaccgacagcgagatgaacaagctgttcgagaagaccaagaagcagctgcgggagaacgccgaggacatgggcaacgggtgcttcaagatctaccacaagtgcgacaacgcctgcatcggcagcatcaggaacgagacatacgaccacaacgtgtacagggacgaggccctgaacaacaggttccagatcaagggcgtggagctgaagtccggctacaaggactggattctgtggatcagcttcgccatgagctgcttcctgctgtgcatcgccctgctgggcttcatcatgtgggcctgccagaagggcaacatcagatgcaacatttgcatctgataagaattctaggctggagcctcggtggccatgcttcttgccccttgggcctccccccagcccctcctccccttcctgcacccgtacccccgtggtctttgaataaagtctgagtgggcggcactagtaaaaaaaaaaaaaaaaaaaaaaaaaaaaaaaaaaaaaaaaaaaaaaaaaaaaaaaaaaaaaaaaaaaaaaaaaaaaaaaaaaaaaaaaaaaaaaaaaaaaaaaaaaaaaaaaaaaaaaaaaaaaaaaaaaaaaaaaaaaaaaaaaa

SEQ ID NO: 9 - RNA, 1075 nt, synthetic construct
  source 1..1075: mol_type = other RNA
ggggggatccaagcttagcttgcttgttctttttgcagaagctcagaataaacgctcaactttggcgccgccaccatggactggacctggattctgttcctggtggctgccgccaccagggtgcacagcagggtgcagcccaccgagagcatcgtgaggttccccaacatcaccaacctgtgccccttcgacgaggtgttcaacgccaccaggttcgcctccgtgtacgcctggaaccggaagaggatcagcaactgcgtggccgactacagcgtgctgtacaactttgcccccttcttcgccttcaagtgctacggcgtgagccccaccaagctgaacgacctgtgcttcaccaacgtgtacgccgacagcttcgtgatcaggggcaacgaggtgtcccagattgcccccggccagaccgggaacatcgctgactacaactacaagctgcccgatgacttcaccggctgcgtgatcgcctggaacagcaacaagctggacagcaaggtggggggcaactacaattaccggtaccggctgttccggaagagcaacctgaagcctttcgagagggacatcagcacagagatctaccaggccggcaacaagccctgcaacggggtggccggcgtgaactgttacttccccctgcagagctacgggttcaggcccacctacggggtgggccaccagccctacagggtggtggtgctgagcttcgagctgctgcacgcccccgccaccgtgtgtgggcctaagaagagcaccaacctggtgaagaacaagtgcgtgaacttctgataagaattctaggctggagcctcggtggccatgcttcttgccccttgggcctccccccagcccctcctccccttcctgcacccgtacccccgtggtctttgaataaagtctgagtgggcggcactagtaaaaaaaaaaaaaaaaaaaaaaaaaaaaaaaaaaaaaaaaaaaaaaaaaaaaaaaaaaaaaaaaaaaaaaaaaaaaaaaaaaaaaaaaaaaaaaaaaaaaaaaaaaaaaaaaaaaaaaaaaaaaaaaaaaaaaaaaaaaaaaaaaa

SEQ ID NO: 10 - RNA, 1023 nt, synthetic construct
  source 1..1023: mol_type = other RNA
atgggcggcgcatgagagaagcccagacttgttctttttgcagaagctcagaataaacgctcaactttggcgccgccaccatggtgagcaagggcgaggagctgttcaccggggtggtgcccatcctggtcgagctggacggcgacgtaaacggccacaagttcagcgtgtccggcgagggcgagggcgatgccacctacggcaagctgaccctgaagttcatctgcaccaccggcaagctgcccgtgccctggcccaccctcgtgaccaccctgacctacggcgtgcagtgcttcagccgctaccccgaccacatgaagcagcacgacttcttcaagtccgccatgcccgaaggctacgtccaggagcgcaccatcttcttcaaggacgacggcaactacaagacccgcgccgaggtgaagttcgagggcgacaccctggtgaaccgcatcgagctgaagggcatcgacttcaaggaggacggcaacatcctggggcacaagctggagtacaactacaacagccacaacgtctatatcatggccgacaagcagaagaacggcatcaaggtgaacttcaagatccgccacaacatcgaggacggcagcgtgcagctcgccgaccactaccagcagaacacccccatcggcgacggccccgtgctgctgcccgacaaccactacctgagcacccagtccgccctgagcaaagaccccaacgagaagcgcgatcacatggtcctgctggagttcgtgaccgccgccgggatcactctcggcatggacgagctgtacaagtgataagaattctaggctggagcctcggtggccatgcttcttgccccttgggcctccccccagcccctcctccccttcctgcacccgtacccccgtggtctttgaataaagtctgagtgggcggcactagtaaaaaaaaaaaaaaaaaaaaaaaaaaaaaaaaaaaaaaaaaaaaaaaaaaaaaaaaaaaaaaaaaaaaaaaaaaaaaaaaaaaaaaaaaaaaaaa

SEQ ID NO: 11 - RNA, 1927 nt, synthetic construct
  source 1..1927: mol_type = other RNA
atggggatccaagcttagcttgcttgttctttttgcagaagctcagaataaacgctcaactttggcgccgccaccatggagctgctgatcctgaaggctaatgccattaccaccattctgaccgccgtgacattctgcttcgcgagcgggcagaacatcaccgaggagttctaccagagcacctgttctgccgtcagcaaggggtacctgtccgccctgcggacaggatggtatacctcagtgatcacaattgagctgtccaatattaaggagaataagtgcaatgggactgacgccaaggtgaagctgatcaagcaggagctggacaagtacaagaacgccgtgacagagctgcagctgctcatgcagagcacccccgccaccgggagtggcagcgccatctgcagcggcgtggccgtctgcaaggtgctgcacctcgagggcgaggtgaataagatcaagagtgctctgctgagcactaacaaggctgtcgtgtctctgtccaacggcgtgtctgtgctgaccttcaaggtcctggacctgaagaattacattgacaagcagctcctgcccatcctgaacaagcagagctgttctatctccaatattgagacagttatcgagtttcagcagaagaacaacaggctgcttgagatcacacgggagttcagcgtgaacgctggggtgaccactcccgtgtccacttacatgctgaccaactcagagctgctgtccctgatcaacgacatgcctattacaaacgaccagaagaagttgatgagcaacaacgtgcagatcgtgagacagcagtcttacagcatcatgtgcatcatcaaggaggaggtgctggcgtacgtggtgcagctgcccctgtatggggtcatcgacaccccttgttggaagctgcacacttctcccctgtgcacgaccaatacgaaggagggcagcaacatctgtctgacccggacagatcggggctggtattgcgacaatgccggctccgtgtccttcttcccccaggctgagacttgcaaggtgcagagtaaccgggtgttctgcgacaccatgaactcccggactctgccctccgaggtgaacctgtgcaacgtggacattttcaaccccaagtacgattgcaagatcatgactagcaagaccgacgtgtcttctagcgtgattaccagcctgggggcgattgtgtcgtgctacgggaagacgaagtgtacagcttccaacaagaacaggggcatcatcaagaccttctctaatgggtgcgactacgtcagcaataagggcgtcgacaccgtcagcgtggggaacaccttgtactgcgtgaacaagcaggagggcaagagcctgtacgtgaagggggagcccattatcaacttctacgaccccctggtgttccccagcgacgagttcgacgcctctatcagccaggtgaacgagaagatcaatcagtccctggccttcattaggaagtctgatgagctgctgcacaacgtgaacgccgggaagagcactacgaatatcatgatcacgacgatcatcatcgtgatcattgtgatcctgctcagcctgatcgccgtggggctgctcctgtactgcaaggccaggagcacccccgtgaccctgtccaaggatcagctgagcgggatcaacaatatcgctttcagcaactgataagaattctaggctggagcctcggtggccatgcttcttgccccttgggcctccccccagcccctcctccccttcctgcacccgtacccccgtggtctttgaataaagtctgagtgggcggcactagtaaaaaaaaaaaaaaaaaaaaaaaaaaaaaaaaaaaaaaaaaaaaaaaaaaaaaaaaaaaaaaaaaaaaaaaaaaaaaaaaaaaaaaaaaaaaaaaaaaaaaaaaaaaaaaaaaaaa

SEQ ID NO: 12 - RNA, 1023 nt, synthetic construct; identical to SEQ ID NO: 10
  source 1..1023: mol_type = other RNA

SEQ ID NO: 13 - RNA, 1026 nt, synthetic construct
  source 1..1026: mol_type = other RNA
atgaaataaggatccttgttctttttgcagaagctcagaataaacgctcaactttggcgccgccaccatggactggacctggatactgttcctggtggccgccgccaccagagtgcacagccgggtccagccaaccgagagcatcgtgagattccccaacataacaaacctgtgccccttcgacgaggtgttcaacgccaccagattcgccagcgtgtacgcctggaacagaaaaagaatcagcaactgcgtggccgactacagcgtgctgtacaacttcgcccccttcttcgccttcaaatgctacggcgtgagcccaaccaaactgaacgacctgtgcttcaccaacgtgtacgccgacagcttcgtgatcagaggcaacgaggtgagccagatcgccccaggccagaccggaaacatcgccgactacaactacaaactgcccgacgacttcaccggctgcgtgatcgcctggaacagcaacaaactggacagcaaagtgggaggcaactacaactacagatacagactgttcagaaaaagcaacctgaaacccttcgagcgagacatcagcaccgaaatctaccaggccggcaacaaaccctgcaacggcgtggccggggtgaactgctacttccccctgcagagctacggattcagacccacctacggcgtggggcaccagccctaccgggtggtggtcctgagcttcgagctgctgcacgcccccgcaaccgtgtgcggccccaaaaaatcgaccaacctggtgaaaaacaaatgcgtgaacttctgataagaattctaggctggagcctcggtggccatgcttcttgccccttgggcctccccccagcccctcctccccttcctgcacccgtacccccgtggtctttgaataaagtctgagtgggcggcactagtaaaaaaaaaaaaaaaaaaaaaaaaaaaaaaaaaaaaaaaaaaaaaaaaaaaaaaaaaaaaaaaaaaaaaaaaaaaaaaaaaaaaaaaaaaaaaaaaaaaaaaaaa

SEQ ID NO: 14 - RNA, 1894 nt, synthetic construct
  source 1..1894: mol_type = other RNA
atggggatccaagcttagcttgcttgttctttttgcagaagctcagaataaacgctcaactttggcgccgccaccatggtgcctcaggccctgttgtttgtgccactgctgggctttagcctgtgttttggcaaattcccaatctacaccatccccgatgagctgggcccttggagccctatcgacatccaccatctcagctgccccaacaacctggtggtggaagatgagggctgcaccaatctgagcgagttcagctacatggaactgaaggtgggctatatcagcgccatcaaggtgaacggcttcacctgtacaggcgtcgtgaccgaggctgagacatacaccaacttcgtgggatacgtgacaaccaccttcaagagaaagcacttcaggccaacacctgacgcctgcagagccgcctacaactggaagatggccggcgatccacggtacgaggaaagcctgcacaacccttatcctgattaccactggctgagaacagtgcggacaacaaaggaaagcctgattattatcagccccagcgtgaccgacctggacccttacgacaagtctctgcacagcagagtgtttcctggagggaagtgctccggcatcaccgtgtcctctacctactgcagcaccaatcacgactacaccatctggatgcctgagaaccccagacccagaaccccttgcgacatcttcaccaacagccgcggaaaacgcgcttctaagggcaacaagacatgcggcttcgtcgacgagagaggcctgtacaagagcctaaaaggcgcttgtagactgaagctgtgcggcgtgttaggcctgagactgatggacggcacgtgggtcgccatgcagaccagcgacgagacaaagtggtgccctcctgatcagctggtgaacctgcatgatttccggagcgacgagatcgagcacctggtggtggaagaacttgttaagaagcgggaagagtgcctggacgccctggaaagcatcatgaccaccaagtccgtgtccttcagacggctgagccacctgcggaaactggttcctggcttcggcaaggcctataccatcttcaacaagacactgatggaagccgacgctcactacaagagcgttagaacctggaacgagattatcccttctaagggctgtctgaaagtgggcggcagatgccacccccacgtgaatggcgtgttcttcaacggcatcatcctgggacctgatggccacgtgctgatccccgagatgcaaagcagcctgctgcagcaacacatggaactgctgaagtcctctgtgatcccactgatgcaccctctggccgatcctagcaccgtgttcaaggaaggcgacgaggccgaggacttcgtggaggtgcacctgcctgacgtgtacaagcagatctctggcgtggacctgggactgcccaattggggaaaatacgtgctgatgaccgccggagccatgatcggcctggtgctgatctttagcctgatgacatggtgtcggagagccaaccggcctgagtccaagcagagaagcttcggcggcaccggcagaaacgtgtctgtgaccagccagtctggcaaggtgatccccagctgggagtcttacaaatctggcggacagacaagactgtgataagaattctaggctggagcctcggtggccatgcttcttgccccttgggcctccccccagcccctcctccccttcctgcacccgtacccccgtggtctttgaataaagtctgagtgggcggcactagtaaaaaaaaaaaaaaaaaaaaaaaaaaaaaaaaaaaaaaaaaaaaaaaaaaaaaaaaaaaaaaaaaaaaaaaaaaaaaaaaaaaaaaaaaaaaaaaaaaaaaaaaaaaaaaaaaaaa

SEQ ID NO: 15 - RNA, 1894 nt, synthetic construct
  source 1..1894: mol_type = other RNA
atggggatccaagcttagcttgcttgttctttttgcagaagctcagaataaacgctcaactttggcgccgccaccatggtgccgcaggccctcctgttcgtgcccctgctgggattttccctttgcttcgggaagttcccaatctatacgatccccgacgagctcgggccgtggagccccatcgacatccaccacctgagttgtcccaacaacttggtggtggaggatgagggctgcacgaacctctctgagttcagctacatggagctgaaggtggggtacatctccgccatcaaggtcaacggcttcacgtgcacgggagtcgtgaccgaggcggagacgtacaccaacttcgttgggtacgtgaccaccaccttcaagaggaagcattttcggcccacgcccgacgcttgtcgggcggcgtataattggaagatggccggggaccctcggtacgaggagtccctgcacaatccttaccctgactaccactggctgcggactgtgaggaccacgaaggagtcactgatcatcatttcgcccagtgtcaccgatctggacccgtacgacaagtcactgcactccagggtgttccctggaggcaagtgctccgggatcacagtgagcagcacgtactgcagcaccaaccacgactataccatctggatgccagagaatcctcggcctcgtaccccctgcgacatctttacaaacagtcgggggaagcgggcgagcaaggggaacaagacctgcggcttcgtggatgagcgcggcctgtacaagagcctgaagggggcttgccgtctgaagctgtgtggcgtgctcgggctccgtctgatggacgggacctgggtcgccatgcagacttcagacgagacaaagtggtgccctcccgaccagctggtcaatctccacgacttcaggtccgatgagatcgagcacctggtcgtggaggagctcgtcaagaagcgcgaggagtgcctcgacgctcttgagagcatcatgaccaccaagagcgtcagcttccgcaggctgagccacctgcggaagctggtgcctgggttcgggaaggcctacaccatcttcaacaagaccctgatggaggccgacgcgcactacaagagcgtgcggacctggaatgagatcattccatccaagggctgtctgaaggtgggtgggcggtgccacccacacgtcaacggcgtgttcttcaacgggatcatcctcgggcctgacgggcacgtgctcatcccggagatgcagagctcgctgctccagcagcacatggagctgctgaagagcagcgtgattcccctgatgcatccgctcgctgatccctcgactgtgtttaaggagggggacgaggccgaggatttcgtggaggtccacctccctgacgtctacaagcagatcagcggggtggaccttgggctcccaaactggggcaagtacgtgctgatgacagccggggccatgatcggcctcgtgctgatcttctcactgatgacctggtgtcggcgggccaatcggcccgagagcaagcagcgctctttcgggggcactgggcggaatgtgtcagtgacttctcagtccgggaaggtgataccttcctgggagtcctacaagtccggcggccagacgcggctgtgataagaattctaggctggagcctcggtggccatgcttcttgccccttgggcctccccccagcccctcctccccttcctgcacccgtacccccgtggtctttgaataaagtctgagtgggcggcactagtaaaaaaaaaaaaaaaaaaaaaaaaaaaaaaaaaaaaaaaaaaaaaaaaaaaaaaaaaaaaaaaaaaaaaaaaaaaaaaaaaaaaaaaaaaaaaaaaaaaaaaaaaaaaaaaaaaaa

SEQ ID NO: 16 - RNA, 1894 nt, synthetic construct
  source 1..1894: mol_type = other RNA
atggggatccctgaactgggttaggtgccgctgttgctgctcgtgttgaatctagaaccgtagccagacgccaccatggtgccgcaggccctcctgttcgtgcccctgctgggattttccctttgcttcgggaagttcccaatctatacgatccccgacgagctcgggccgtggagccccatcgacatccaccacctgagttgtcccaacaacttggtggtggaggatgagggctgcacgaacctctctgagttcagctacatggagctgaaggtggggtacatctccgccatcaaggtcaacggcttcacgtgcacgggagtcgtgaccgaggcggagacgtacaccaacttcgttgggtacgtgaccaccaccttcaagaggaagcattttcggcccacgcccgacgcttgtcgggcggcgtataattggaagatggccggggaccctcggtacgaggagtccctgcacaatccttaccctgactaccactggctgcggactgtgaggaccacgaaggagtcactgatcatcatttcgcccagtgtcaccgatctggacccgtacgacaagtcactgcactccagggtgttccctggaggcaagtgctccgggatcacagtgagcagcacgtactgcagcaccaaccacgactataccatctggatgccagagaatcctcggcctcgtaccccctgcgacatctttacaaacagtcgggggaagcgggcgagcaaggggaacaagacctgcggcttcgtggatgagcgcggcctgtacaagagcctgaagggggcttgccgtctgaagctgtgtggcgtgctcgggctccgtctgatggacgggacctgggtcgccatgcagacttcagacgagacaaagtggtgccctcccgaccagctggtcaatctccacgacttcaggtccgatgagatcgagcacctggtcgtggaggagctcgtcaagaagcgcgaggagtgcctcgacgctcttgagagcatcatgaccaccaagagcgtcagcttccgcaggctgagccacctgcggaagctggtgcctgggttcgggaaggcctacaccatcttcaacaagaccctgatggaggccgacgcgcactacaagagcgtgcggacctggaatgagatcattccatccaagggctgtctgaaggtgggtgggcggtgccacccacacgtcaacggcgtgttcttcaacgggatcatcctcgggcctgacgggcacgtgctcatcccggagatgcagagctcgctgctccagcagcacatggagctgctgaagagcagcgtgattcccctgatgcatccgctcgctgatccctcgactgtgtttaaggagggggacgaggccgaggatttcgtggaggtccacctccctgacgtctacaagcagatcagcggggtggaccttgggctcccaaactggggcaagtacgtgctgatgacagccggggccatgatcggcctcgtgctgatcttctcactgatgacctggtgtcggcgggccaatcggcccgagagcaagcagcgctctttcgggggcactgggcggaatgtgtcagtgacttctcagtccgggaaggtgataccttcctgggagtcctacaagtccggcggccagacgcggctgtgataagaattctaggctggagcctcggtggccatgcttcttgccccttgggcctccccccagcccctcctccccttcctgcacccgtacccccgtggtctttgaataaagtctgagtgggcggcactagtaaaaaaaaaaaaaaaaaaaaaaaaaaaaaaaaaaaaaaaaaaaaaaaaaaaaaaaaaaaaaaaaaaaaaaaaaaaaaaaaaaaaaaaaaaaaaaaaaaaaaaaaaaaaaaaaaaaa

SEQ ID NO: 17 - RNA, 1894 nt, synthetic construct
  source 1..1894: mol_type = other RNA
atggggatccctgaactgggttaggtgccgctgttgctgctcgtgttgaatctagaaccgtagccagacgccaccatggtgccccaggccctgctgttcgtgcctctgctgggattcagcctgtgcttcgggaagttcccaatttacaccatccccgatgagctgggcccttggtcccccatcgacatccaccacctgagttgccccaacaatctggtggtggaggatgaggggtgcaccaacctgagcgagttcagctacatggagctgaaggtggggtacatctctgccatcaaggtgaacggcttcacctgcaccggcgtggtgactgaggcagagacatacaccaacttcgtgggctatgtgaccaccaccttcaagcggaagcacttcaggcccacccccgacgcctgccgcgccgcctataactggaagatggccggggaccctcggtacgaggagtccctgcacaatccttacccagattatcactggctgcggacagtgcggaccaccaaggagtctctgatcatcatcagccctagcgtgacagacctggacccttacgataagagcctgcacagcagggtgttccccggcggcaagtgcagcggcatcaccgtgtccagcacctactgcagcaccaaccacgactacaccatctggatgccagagaaccccaggccccgcaccccctgcgacatcttcacaaattccagggggaagcgggcctccaagggcaataagacttgcgggttcgtggatgagcggggcctgtacaagtccctgaagggggcttgcaggctgaagctgtgcggggtgctgggcctgaggctgatggacggcacctgggtcgccatgcagacctcagacgagacaaagtggtgccctcctgaccagctggtgaacctgcacgacttcaggagcgatgagatcgagcacctggtggtggaggagctcgtgaagaagagggaggagtgcctggacgctctggagtccatcatgactaccaagagcgtcagcttccgcaggctgagccacctgcggaagctggtgccaggcttcggcaaggcctacaccatcttcaacaagaccctgatggaggccgacgctcactacaagagcgtgcggacctggaatgagatcattccatccaagggctgtctgaaggtgggaggccgctgccacccccacgtcaacggcgtgttcttcaacgggatcatcctggggcctgacgggcacgtgctgatcccagagatgcagagcagcctgctgcagcagcacatggagctgctgaagtccagcgtgatcccactgatgcatcccctggccgacccctcaactgtgttcaaggagggggacgaggccgaggacttcgtggaggtccacctgcctgacgtgtacaagcagatcagcggcgtggacctggggctgcccaactggggcaagtacgtgctgatgaccgccggcgccatgatcggtctggtgctgatcttcagcctgatgacatggtgccggcgggccaaccggcccgagagcaagcagcgctctttcgggggcaccggccggaacgtgtccgtgacctcccagtctgggaaggtgatccccagctgggagagctacaagtccggcggccagacccggctgtgataagaattctaggctggagcctcggtggccatgcttcttgccccttgggcctccccccagcccctcctccccttcctgcacccgtacccccgtggtctttgaataaagtctgagtgggcggcactagtaaaaaaaaaaaaaaaaaaaaaaaaaaaaaaaaaaaaaaaaaaaaaaaaaaaaaaaaaaaaaaaaaaaaaaaaaaaaaaaaaaaaaaaaaaaaaaaaaaaaaaaaaaaaaaaaaaaa

SEQ ID NO: 18 - RNA, 2002 nt, synthetic construct
  source 1..2002: mol_type = other RNA
agggggatccaagcttagcttgcttgttctttttgcagaagctcagaataaacgctcaactttggcgccgccaccatggaggacgccaaaaacatcaaaaaaggccccgcccccttctaccccctggaggacggcaccgccggagagcagctgcacaaagccatgaaaagatacgccctggtccccggcaccatcgccttcaccgacgcccacatcgaggtggacatcacctacgccgagtacttcgagatgagcgtgagactggccgaagccatgaaaaggtacggcctgaacacaaaccacagaatcgtggtgtgcagcgagaacagcctgcagttcttcatgcccgtgctgggagccctgttcatcggcgtggccgtggcccccgccaacgacatctacaacgagagagagctgctcaacagcatgggcatcagccagcccaccgtggtgttcgtgagcaaaaaaggcctgcagaaaatcctgaacgtgcagaaaaaactccccatcatccagaaaatcatcatcatggatagcaaaaccgactaccagggcttccagagcatgtacaccttcgtgaccagccacctgccccctggcttcaacgagtacgacttcgtgccggagagcttcgacagggacaaaaccatcgccctgatcatgaacagcagcggcagcaccggcctgcccaaaggcgtggccctgccccaccggacagcctgcgtgagattcagccacgccagagatcccatcttcggcaaccagatcatccccgacaccgccatcctgagcgtggtcccattccaccacggcttcggcatgttcaccaccctgggctacctgatctgcggcttccgcgtggtgctgatgtacagattcgaggaggagctgttcctaagaagtctgcaggactacaaaatccagagcgccctgctggtgcccaccctgttcagcttcttcgccaaaagcaccctgatcgacaaatacgacctgagcaacctgcacgagatcgccagcggcggcgccccactgagcaaagaggtgggcgaggccgtggccaaaagattccacctgcccggaatcagacagggctacggcctgacggaaaccaccagcgccatcctgatcacccccgagggcgacgacaaacccggcgccgtgggcaaagtggtgcccttcttcgaggccaaagtggtggacctggacaccggcaaaaccctgggagtgaaccagagaggggagctgtgcgtgagaggccccatgatcatgagcggctacgtgaacaaccccgaggccaccaacgccctcatcgacaaagacggctggctgcacagcggcgacatcgcctactgggacgaggacgagcacttcttcatcgtggaccgcctgaaatcgctgatcaaatacaaaggataccaggtggcccccgccgagctggagagcatcctgctgcagcaccccaacatcttcgacgccggcgtggccggcctgcccgacgacgacgccggcgagctgcccgccgccgtcgtggtgctggagcacggaaaaaccatgaccgagaaagagatcgtggactacgtggccagccaggtgaccacagccaaaaaactgaggggcggcgtggtgttcgtggacgaggtgcccaaaggcctgaccggcaaactggacgcccggaaaatcagagagatcctgatcaaagccaaaaaaggcggcaaaatcgccgtgtgataagaattctaggctggagcctcggtggccatgcttcttgccccttgggcctccccccagcccctcctccccttcctgcacccgtacccccgtggtctttgaataaagtctgagtgggcggcactagtaaaaaaaaaaaaaaaaaaaaaaaaaaaaaaaaaaaaaaaaaaaaaaaaaaaaaaaaaaaaaaaaaaaaaaaaaaaaaaaaaaaaaaaaaaaaaaaaaaaaaaaaaaaaaaaaaaaaaaaaaaaaaaaaaaaaaaaaaaaaaaaaaa

SEQ ID NO: 19 - RNA, 1019 nt, synthetic construct
  source 1..1019: mol_type = other RNA
aggatccttgttctttttgcagaagctcagaataaacgctcaactttggcgccgccaccatggactggacctggatactgttcctggtggccgccgccaccagagtgcacagccgggtccagccaaccgagagcatcgtgagattccccaacataacaaacctgtgccccttcgacgaggtgttcaacgccaccagattcgccagcgtgtacgcctggaacagaaaaagaatcagcaactgcgtggccgactacagcgtgctgtacaacttcgcccccttcttcgccttcaaatgctacggcgtgagcccaaccaaactgaacgacctgtgcttcaccaacgtgtacgccgacagcttcgtgatcagaggcaacgaggtgagccagatcgccccaggccagaccggaaacatcgccgactacaactacaaactgcccgacgacttcaccggctgcgtgatcgcctggaacagcaacaaactggacagcaaagtgggaggcaactacaactacagatacagactgttcagaaaaagcaacctgaaacccttcgagcgagacatcagcaccgaaatctaccaggccggcaacaaaccctgcaacggcgtggccggggtgaactgctacttccccctgcagagctacggattcagacccacctacggcgtggggcaccagccctaccgggtggtggtcctgagcttcgagctgctgcacgcccccgcaaccgtgtgcggccccaaaaaatcgaccaacctggtgaaaaacaaatgcgtgaacttctgataagaattctaggctggagcctcggtggccatgcttcttgccccttgggcctccccccagcccctcctccccttcctgcacccgtacccccgtggtctttgaataaagtctgagtgggcggcactagtaaaaaaaaaaaaaaaaaaaaaaaaaaaaaaaaaaaaaaaaaaaaaaaaaaaaaaaaaaaaaaaaaaaaaaaaaaaaaaaaaaaaaaaaaaaaaaaaaaaaaaaaaa

SEQ ID NO: 20 - RNA, 901 nt, synthetic construct
  source 1..901: mol_type = other RNA
agggggatccaagcttagcttgcttgttctttttgcagaagctcagaataaacgctcaactttggcgccgccaccatgggtgtgcatgagtgtcccgcttggctttggctgttattatcattactttccttacctcttggcctgcctgtcttaggcgcccctcctcgtttaatctgtgatagccgtgtgttagagagatacttgcttgaggctaaagaggccgagaatattactaccggttgtgctgaacattgctcgctgaacgagaacattaccgtgcccgacaccaaagttaacttctatgcttggaaacgtatggaggtgggtcagcaggccgttgaggtatggcagggtttggcccttctttcggaggccgtgttacgtggtcaggctctcttggttaactcttctcagccttgggagcctttacagttacatgttgataaagccgttagcggcttgagaagtttgaccactttgcttcgggctctgggtgctcaaaaagaggctatttcaccccctgatgctgctagcgctgctccacttagaaccatcactgccgacacttttcgtaaattgtttcgtgtttatagcaatttcttacgtggcaaactgaaattatacactggcgaggcttgcagaactggtgacagatgataagaattctaggctggagcctcggtggccatgcttcttgccccttgggcctccccccagcccctcctccccttcctgcacccgtacccccgtggtctttgaataaagtctgagtgggcggcactagtaaaaaaaaaaaaaaaaaaaaaaaaaaaaaaaaaaaaaaaaaaaaaaaaaaaaaaaaaaaaaaaaaaaaaaaaaaaaaaaaaaaaaaaaaaaaaaaaaaaaaaaaaaaaaaaaaaaa